European Patent Specification EP 3 487 528 B1, published August 30, 2023. Title: Surface decoration of extracellular vesicles. Applicant: Evox Therapeutics Ltd. The sequence listing filed with the application follows.

SEQUENCE LISTING (83 sequences)

SEQ ID NO: 1 - protein, 227 aa, Homo sapiens
PVKGGTKCIKYLLFGFNFIFWLAGIAVLAIGLWLRFDSQTKSIFEQETNNNNSSFYTGVYILIGAGALMMLVGFLGCCGAVQESQCMLGLFFGFLLVIFAIEIAAAIWGYSHKDEVIKEVQEFYKDTYNKLKTKDEPQRETLKAIHYALNCCGLAGGVEQFISDICPKKDVLETFTVKSCPDAIKEVFDNKFHIIGAVGIGIAVVMIFGMIFSMILCCAIRRNREMV

SEQ ID NO: 2 - protein, 219 aa, Homo sapiens
MGMSSLKLLKYVLFFFNLLFWICGCCILGFGIYLLIHNNFGVLFHNLPSLTLGNVFVIVGSIIMVVAFLGCMGSIKENKCLLMSFFILLLIILLAEVTLAILLFVYEQKLNEYVAKGLTDSIHRYHSDNSTKAAWDSIQSFLQCCGINGTSDWTSGPPASCPSDRKVEGCYAKARLWFHSNFLYIGIITICVCVIEVLGMSFALTLNCQIDKTSQTIGL

SEQ ID NO: 3 - protein, 237 aa, Homo sapiens
AVEGGMKCVKFLLYVLLLAFCACAVGLIAVGVGAQLVLSQTIIQGATPGSLLPVVIIAVGVFLFLVAFVGCCGACKENYCLMITFAIFLSLIMLVEVAAAIAGYVFRDKVMSEFNNNFRQQMENYPKNNHTASILDRMQADFKCCGAANYTDWEKIPSMSKNRVPDSCCINVTVGCGINFNEKAIHKEGCVEKIGGWLRKNVLVVAAAALGIAFVEVLGIVFACCLVKSIRSGYEVM

SEQ ID NO: 4 - protein, 236 aa, Homo sapiens
MGVEGCTKCIKYLLFVFNFVFWLAGGVILGVALWLRHDPQTTNLLYLELGDKPAPNTFYVGIYILIAVGAVMMFVGFLGCYGAIQESQCLLGTFFTCLVILFACEVAAGIWGFVNKDQIAKDVKQFYDQALQQAVVDDDANNAKAVVKTFHETLDCCGSSTLTALTTSVLKNNLCPSGSNIISNLFKEDCHQKIDDLFSGKLYLIGIAAIVVAVIMIFEMILSMVLCCGIRNSSVY

SEQ ID NO: 5 - protein, 532 aa, Homo sapiens
MAPSSPRPALPALLVLLGALFPGPGNAQTSVSPSKVILPRGGSVLVTCSTSCDQPKLLGIETPLPKKELLLPGNNRKVYELSNVQEDSQPMCYSNCPDGQSTAKTFLTVYWTPERVELAPLPSWQPVGKNLTLRCQVEGGAPRANLTVVLLRGEKELKREPAVGEPAEVTTTVLVRRDHHGANFSCRTELDLRPQGLELFENTSAPYQLQTFVLPATPPQLVSPRVLEVDTQGTVVCSLDGLFPVSEAQVHLALGDQRLNPTVTYGNDSFSAKASVSVTAEDEGTQRLTCAVILGNQSQETLQTVTIYSFPAPNVILTKPEVSEGTEVTVKCEAHPRAKVTLNGVPAQPLGPRAQLLLKATPEDNGRSFSCSATLEVAGQLIHKNQTRELRVLYGPRLDERDCPGNWTWPENSQQTPMCQAWGNPLPELKCLKDGTFPLPIGESVTVTRDLEGTYLCRARSTQGEVTRKVTVNVLSPRYEIVIITVVAAAVIMGTAGLSTYLYNRQRKIKKYRLQQAQKGTPMKPNTQATPP

SEQ ID NO: 6 - protein, 547 aa, Homo sapiens
MATMVPSVLWPRACWTLLVCCLLTPGVQGQEFLLRVEPQNPVLSAGGSLFVNCSTDCPSSEKIALETSLSKELVASGMGWAAFNLSNVTGNSRILCSVYCNGSQITGSSNITVYRLPERVELAPLPPWQPVGQNFTLRCQVEDGSPRTSLTVVLLRWEEELSRQPAVEEPAEVTATVLASRDDHGAPFSCRTELDMQPQGLGLFVNTSAPRQLRTFVLPVTPPRLVAPRFLEVETSWPVDCTLDGLFPASEAQVYLALGDQMLNATVMNHGDTLTATATATARADQEGAREIVCNVTLGGERREARENLTVFSFLGPIVNLSEPTAHEGSTVTVSCMAGARVQVTLDGVPAAAPGQPAQLQLNATESDDGRSFFCSATLEVDGEFLHRNSSVQLRVLYGPKIDRATCPQHLKWKDKTRHVLQCQARGNPYPELRCLKEGSSREVPVGIPFFVNVTHNGTYQCQASSSRGKYTLVVVMDIEAGSSHFVPVFVAVLLTLGVVTIVLALMYVFREHQRSGSYHVREESTYLPLTSMQPTEAMGEEPSRAE

SEQ ID NO: 7 - protein, 427 aa, Homo sapiens
MFFTCGPNEAMVVSGFCRSPPVMVAGGRVFVLPCIQQIQRISLNTLTLNVKSEKVYTRHGVPISVTGIAQVKIQGQNKEMLAAACQMFLGKTEAEIAHIALETLEGHQRAIMAHMTVEEIYKDRQKFSEQVFKVASSDLVNMGISVVSYTLKDIHDDQDYLHSLGKARTAQVQKDARIGEAEAKRDAGIREAKAKQEKVSAQYLSEIEMAKAQRDYELKKAAYDIEVNTRRAQADLAYQLQVAKTKQQIEEQRVQVQVVERAQQVAVQEQEIARREKELEARVRKPAEAERYKLERLAEAEKSQLIMQAEAEAASVRMRGEAEAFAIGARARAEAEQMAKKAEAFQLYQEAAQLDMLLEKLPQVAEEISGPLTSANKITLVSSGSGTMGAAKVTGEVLDILTRLPESVERLTGVSISQVNHKPLRTA

SEQ ID NO: 8 - protein, 427 aa, Homo sapiens
GNCHTVGPNEALVVSGGCCGSDYKQYVFGGWAWAWWCISDTQRISLEIMTLQPRCEDVETAEGVALTVTGVAQVKIMTEKELLAVACEQFLGKNVQDIKNVVLQTLEGHLRSILGTLTVEQIYQDRDQFAKLVREVAAPDVGRMGIEILSFTIKDVYDKVDYLSSLGKTQTAVVQRDADIGVAEAERDAGIREAECKKEMLDVKFMADTKIADSKRAFELQKSAFSEEVNIKTAEAQLAYELQGAREQQKIRQEEIEIEVVQRKKQIAVEAQEILRTDKELIATVRRPAEAEAHRIQQIAEGEKVKQVLLAQAEAEKIRKIGEAEAAVIEAMGKAEAERMKLKAEAYQKYGDAAKMALVLEALPQIAAKIAAPLTKVDEIVVLSGDNSKVTSEVNRLLAELPASVHALTGVDLSKIPLIKKATGVQV

SEQ ID NO: 9 - protein, 1032 aa, Homo sapiens [sequence omitted]

SEQ ID NO: 10 - protein, 760 aa, Homo sapiens
MMDQARSAFSNLFGGEPLSYTRFSLARQVDGDNSHVEMKLAVDEEENADNNTKANVTKPKRCSGSICYGTIAVIVFFLIGFMIGYLGYCKGVEPKTECERLAGTESPVREEPGEDFPAARRLYWDDLKRKLSEKLDSTDFTGTIKLLNENSYVPREAGSQKDENLALYVENQFREFKLSKVWRDQHFVKIQVKDSAQNSVIIVDKNGRLVYLVENPGGYVAYSKAATVTGKLVHANFGTKKDFEDLYTPVNGSIVIVRAGKITFAEKVANAESLNAIGVLIYMDQTKFPIVNAELSFFGHAHLGTGDPYTPGFPSFNHTQFPPSRSSGLPNIPVQTISRAAAEKLFGNMEGDCPSDWKTDSTCRMVTSESKNVKLTVSNVLKEIKILNIFGVIKGFVEPDHYVVVGAQRDAWGPGAAKSGVGTALLLKLAQMFSDMVLKDGFQPSRSIIFASWSAGDFGSVGATEWLEGYLSSLHLKAFTYINLDKAVLGTSNFKVSASPLLYTLIEKTMQNVKHPVTGQFLYQDSNWASKVEKLTLDNAAFPFLAYSGIPAVSFCFCEDTDYPYLGTTMDTYKELIERIPELNKVARAAAEVAGQFVIKLTHDVELNLDYERYNSQLLSFVRDLNQYRADIKEMGLSLQWLYSARGDFFRATSRLTTDFGNAEKTDRFVMKKLNDRVMRVEYHFLSPYVSPKESPFRHVFWGSGSHTLPALLENLKLRKQNNGAFNETLFRNQLALATWTIQGAANALSGDVWDIDNEF

SEQ ID NO: 11 - protein, 865 aa, Homo sapiens
MALVLGSLLLLGLCGNSFSGGQPSSTDAPKAWNYELPATNYETQDSHKAGPIGILFELVHIFLYVVQPRDFPEDTLRKFLQKAYESKIDYDKPETVILGLKIVYYEAGIILCCVLGLLFIILMPLVGYFFCMCRCCNKCGGEMHQRQKENGPFLRKCFAISLLVICIIISIGIFYGFVANHQVRTRIKRSRKLADSNFKDLRTLLNETPEQIKYILAQYNTTKDKAFTDLNSINSVLGGGILDRLRPNIIPVLDEIKSMATAIKETKEALENMNSTLKSLHQQSTQLSSSLTSVKTSLRSSLNDPLCLVHPSSETCNSIRLSLSQLNSNPELRQLPPVDAELDNVNNVLRTDLDGLVQQGYQSLNDIPDRVQRQTTTVVAGIKRVLNSIGSDIDNVTQRLPIQDILSAFSVYVNNTESYIHRNLPTLEEYDSYWWLGGLVICSLLTLIVIFYYLGLLCGVCGYDRHATPTTRGCVSNTGGVFLMVGVGLSFLFCWILMIIVVLTFVFGANVEKLICEPYTSKELFRVLDTPYLLNEDWEYYLSGKLFNKSKMKLTFEQVYSDCKKNRGTYGTLHLQNSFNISEHLNINEHTGSISSELESLKVNLNIFLLGAAGRKNLQDFAACGIDRMNYDSYLAQTGKSPAGVNLLSFAYDLEAKANSLPPGNLRNSLKRDAQTIKTIHQQRVLPIEQSLSTLYQSVKILQRTGNGLLERVTRILASLDFAQNFITNNTSSVIIEETKKYGRTIIGYFEHYLQWIEFSISEKVASCKPVATALDTAVDVFLCSYIIDPLNLFWFGIGKATVFLLPALIFAVKLAKYYRRMDSEDVYDDVETIPMKNMENGNNGYHKDHVYGIHNPVMTSPSQH

SEQ ID NO: 12 - protein, 310 aa, Homo sapiens
MRRAALWLWLCALALSLQPALPQIVATNLPPEDQDGSGDDSDNFSGSGAGALQDITLSQQTPSTWKDTQLLTAIPTSPEPTGLEATAASTSTLPAGEGPKEGEAVVLPEVEPGLTAREQEATPRPRETTQLPTTHLASTTTATTAQEPATSHPHRDMQPGHHETSTPAGPSQADLHTPHTEDGGPSATERAAEDGASSQLPAAEGSGEQDFTFETSGENTAVVAVEPDRRNQSPVDQGATGASQGLLDRKEVLGGVIAGGLVGLIFAVCLVGFMLYRMKKKDEGSYSLEEPKQANGGAYQKPTKQEEFYA

SEQ ID NO: 13 - protein, 150 aa, Homo sapiens [sequence omitted]

SEQ ID NO: 14 - protein, 867 aa, Homo sapiens
ATFISVQLKKTSEVDLAKPLVKFIQQTYPSGGEEQAQYCRAAEELSKLRRAAVGRPLDKHEGALETLLRYYDQICSIEPKFPFSENQICLTFTWKDAFDKGSLFGGSVKLALASLGYEKSCVLFNCAALASQIAAEQNLDNDEGLKIAAKHYQFASGAFLHIKETVLSALSREPTVDISPDTVGTLSLIMLAQAQEVFFLKATRDKMKDAIIAKLANQAADYFGDAFKQCQYKDTLPKEVFPVLAAKHCIMQANAEYHQSILAKQQKKFGEEIARLQHAAELIKTVASRYDEYVNVKDFSDKINRALAAAKKDNDFIYHDRVPDLKDLDPIGKATLVKSTPVNVPISQKFTDLFEKMVPVSVQQSLAAYNQRKADLVNRSIAQMREATTLANGVLASLNLPAAIEDVSGDTVPQSILTKSRSVIEQGGIQTVDQLIKELPELLQRNREILDESLRLLDEEEATDNDLRAKFKERWQRTPSNELYKPLRAEGTNFRTVLDKAVQADGQVKECYQSHRDTIVLLCKPEPELNAAIPSANPAKTMQGSEVVNVLKSLLSNLDEVKKEREGLENDLKSVNFDMTSKFLTALAQDGVINEEALSVTELDRVYGGLTTKVQESLKKQEGLLKNIQVSHQEFSKMKQSNNEANLREEVLKNLATAYDNFVELVANLKEGTKFYNELTEILVRFQNKCSDIVFARKTERDELLKDLQQSIAREPSAPSIPTPAYQSSPAGGHAPTPPTPAPRTMPPTKPQPPARPPPPVLPANRAPSATAPSPVGAGTAAPAPSQTPGSAPPPQAQGPPYPTYPGYPGYCQMPMPMGYNPYAYGQYNMPYPPVYHQSPGQAPYPGPQQPSYPFPQPPQQSYYPQQ

SEQ ID NO: 15 - protein, 297 aa, Homo sapiens
SLYPSLEDLKVDKVIQAQTAFSANPANPAILSEASAPIPHDGNLYPRLYPELSQYMGLSLNEEEIRANVAVVSGAPLQGQLVARPSSINYMVAPVTGNDVGIRRAEIKQGIREVILCKDQDGKIGLRLKSIDNGIFVQLVQANSPASLVGLRFGDQVLQINGENCAGWSSDKAHKVLKQAFGEKITMTIRDRPFERTITMHKDSTGHVGFIFKNGKITSIVKDSSAARNGLLTEHNICEINGQNVIGLKDSQIADILSTSGTVVTITIMPAFIFEHIIKRMAPSIMKSLMDHTIPEV

SEQ ID NO: 16 - protein, 292 aa, Homo sapiens
MSSLYPSLEDLKVDQAIQAQVRASPKMPALPVQATAISPPPVLYPNLAELENYMGLSLSSQEVQESLLQIPEGDSTAVSGPGPGQMVAPVTGYSLGVRRAEIKPGVREIHLCKDERGKTGLRLRKVDQGLFVQLVQANTPASLVGLRFGDQLLQIDGRDCAGWSSHKAHQVVKKASGDKIVVVVRDRPFQRTVTMHKDSMGHVGFVIKKGKIVSLVKGSSAARNGLLTNHYVCEVDGQNVIGLKDKKIMEILATAGNVVTLTIIPSVIYEHMVKKLPPVLLHHTMDHSIPDA

SEQ ID NO: 17 - protein, 410 aa, Homo sapiens
MVCFRLFPVPGSGLVLVCLVLGAVRSYALELNLTDSENATCLYAKWQMNFTVRYETTNKTYKTVTISDHGTVTYNGSICGDDQNGPKIAVQFGPGFSWIANFTKAASTYSIDSVSFSYNTGDNTTFPDAEDKGILTVDELLAIRIPLNDLFRCNSLSTLEKNDVVQHYWDVLVQAFVQNGTVSTNEFLCDKDKTSTVAPTIHTTVPSPTTTPTPKEKPEAGTYSVNNGNDTCLLATMGLQLNITQDKVASVININPNTTHSTGSCRSHTALLRLNSSTIKYLDFVFAVKNENRFYLKEVNISMYLVNGSVFSIANNNLSYWDAPLGSSYMCNKEQTVSVSGAFQINTFDLRVQPFNVTQGKYSTAQDCSADDDNFLVPIAVGAALAGVLILVLLAYFIGLKHHHAGYEQF

SEQ ID NO: 18 - protein, 918 aa, Homo sapiens [sequence omitted]

SEQ ID NO: 19 - protein, 455 aa, Homo sapiens
MGLSTVPDLLLPLVLLELLVGIYPSGVIGLVPHLGDREKRDSVCPQGKYIHPQNNSICCTKCHKGTYLYNDCPGPGQDTDCRECESGSFTASENHLRHCLSCSKCRKEMGQVEISSCTVDRDTVCGCRKNQYRHYWSENLFQCFNCSLCLNGTVHLSCQEKQNTVCTCHAGFFLRENECVSCSNCKKSLECTKLCLPQIENVKGTEDSGTTVLLPLVIFFGLCLLSLLFIGLMYRYQRWKSKLYSIVCGKSTPEKEGELEGTTTKPLAPNPSFSPTPGFTPTLGFSPVPSSTFTSSSTYTPGDCPNFAAPRREVAPPYQGADPILATALASDPIPNPLQKWEDSAHKPQSLDTDDPATLYAVVENVPPLRWKEFVRRLGLSDHEIDRLELQNGRCLREAQYSMLATWRRRTPRREATLELLGRVLRDMDLLGCLEDIEEALCGPAALPPAPSLLR

SEQ ID NO: 20 - protein, 201 aa, Homo sapiens
MRRAWILLTLGLVACVSAESRAELTSDKDMYLDNSSIEEASGVYPIDDDDYASASGSGADEDVESPELTTSRPLPKILLTSAAPKVETTTLNIQNKIPAQTKSPEETDKEKVHLSDSERKMDPAEEDTNVYTEKHSDSLFKRTEVLAAVIAGGVIGFLFAIFLILLLVYRMRKKDEGSYDLGERKPSSAAYQKAPTKEFYA

SEQ ID NO: 21 - protein, 442 aa, Homo sapiens
MKPGPPHRAGAAHGAGAGAGAAAGPGARGLLLPPLLLLLLAGRAAGAQRWRSENFERPVDLEGSGDDDSFPDDELDDLYSGSGSGYFEQESGIETAMRFSPDVALAVSTTPAVLPTTNIQPVGTPFEELPSERPTLEPATSPLVVTEVPEEPSQRATTVSTTMATTAATSTGDPTVATVPATVATATPSTPAAPPFTATTAVIRTTGVRRLLPLPLTTVATARATTPEAPSPPTTAAVLDTEAPTPRLVSTATSRPRALPRPATTQEPDIPERSTLPLGTTAPGPTEVAQTPTPETFLTTIRDEPEVPVSGGPSGDFELPEEETTQPDTANEVVAVGGAAAKASSPPGTLPKGARPGPGLLDNAIDSGSSAAQLPQKSILERKEVLVAVIVGGVVGALFAAFLVTLLIYRMKKKDEGSYTLEEPKQASVTYQKPDKQEEFYA

SEQ ID NO: 22 - protein, 198 aa, Homo sapiens
MAPARLFALLLFFVGGVAESIRETEVIDPQDLLEGRYFSGALPDDEDVVGPGQESDDFELSGSGDLDDLEDSMIGPEVVHPLVPLDNHIPERAGSGSQVPTEPKKLEENEVIPKRISPVEESEDVSNKVSMSSTVQGSNIFERTEVLAALIVGGIVGILFAVFLILLLMYRMKKKDEGSYDLGKKPIYKKAPTNEFYA

SEQ ID NO: 23 - protein, 59 aa, Homo sapiens
MDQARSAFSNLFGGEPLSYTRFSLARQVDGDNSHVEMKLAVDEEENADNNTKANVTKPK

SEQ ID NO: 24 - protein, 267 aa, Homo sapiens
MGSACIKVTKYFLFLFNLIFFILGAVILGFGVWILADKSSFISVLQTSSSSLRMGAYVFIGVGAVTMLMGFLGCIGAVNEVRCLLGLYFAFLLLILIAQVTAGALFYFNMGKLKQEMGGIVTELIRDYNSSREDSLQDAWDYVQAQVKCCGWVSFYNWTDNAELMNRPEVTYPCSCEVKGEEDNSLSVRKGFCEAPGNRTQSGNHPEDWPVYQEGCMEKVQAWLQENLGIILGVGVGVAIIELLGMVLSICLCRHVHSEDYSKVPKY

SEQ ID NO: 25 - protein, 387 aa, Homo sapiens
MPRPRLLAALCGALLCAPSLLVALDICSKNPCHNGGLCEEISQEVRGDVFPSYTCTCLKGYAGNHCETKCVEPLGMENGNIANSQIAASSVRVTFLGLQHWVPELARLNRAGMVNAWTPSSNDDNPWIQVNLLRRMWVTGVVTQGASRLASHEYLKAFKVAYSLNGHEFDFIHDVNKKHKEFVGNWNKNAVHVNLFETPVEAQYVRLYPTSCHTACTLRFELLGCELNGCANPLGLKNNSIPDKQITASSSYKTWGLHLFSWNPSYARLDKQGNFNAWVAGSYGNDQWLQVDLGSSKEVTGIITQGARNFGSVQFVASYKVAYSNDSANWTEYQDPRTGSSKIFPGNWDNHSHKKNLFETPILARYVRILPVAWHNRIALRLELLGC

SEQ ID NO: 26 - protein, 556 aa, Homo sapiens [sequence omitted]

SEQ ID NO: 27 - protein, 595 aa, Homo sapiens
MRVLLAALGLLFLGALRAFPQDRPFEDTCHGNPSHYYDKAVRRCCYRCPMGLFPTQQCPQRPTDCRKQCEPDYYLDEADRCTACVTCSRDDLVEKTPCAWNSSRVCECRPGMFCSTSAVNSCARCFFHSVCPAGMIVKFPGTAQKNTVCEPASPGVSPACASPENCKEPSSGTIPQAKPTPVSPATSSASTMPVRGGTRLAQEAASKLTRAPDSPSSVGRPSSDPGLSPTQPCPEGSGDCRKQCEPDYYLDEAGRCTACVSCSRDDLVEKTPCAWNSSRTCECRPGMICATSATNSCARCVPYPICAAETVTKPQDMAEKDTTFEAPPLGTQPDCNPTPENGEAPASTSPTQSLLVDSQASKTLPIPTSAPVALSSTGKPVLDAGPVLFWVILVLVVVVGSSAFLLCHRRACRKRIRQKLHLCYPVQTSQPKLELVDSRPRRSSTQLRSGASVTEPVAEERGLMSQPLMETCHSVGAAYLESLPLQDASPAGGPSSPRDLPEPRVSTEHTNNKIEKIYIMKADTVIVGTVKAELPEGRGLAGPAEPELEEELEADHTPHYPEQETEPPLGSCSDVMLSVEEEGKEDPLPTAASGK

SEQ ID NO: 28 - protein, 532 aa, Homo Sapiens
MPLFLILCLLQGSSFALPQKRPHPRWLWEGSLPSRTHLRAMGTLRPSSPLCWREESSFAAPNSLKGSRLVSGEPGGAVTIQCHYAPSSVNRHQRKYWCRLGPPRWICQTIVSTNQYTHHRYRDRVALTDFPQRGLFVVRLSQLSPDDIGCYLCGIGSENNMLFLSMNLTISAGPASTLPTATPAAGELTMRSYGTASPVANRWTPGTTQTLGQGTAWDTVASTPGTSKTTASAEGRRTPGATRPAAPGTGSWAEGSVKAPAPIPESPPSKSRSMSNTTEGVWEGTRSSVTNRARASKDRREMTTTKADRPREDIEGVRIALDAAKKVLGTIGPPALVSETLAWEILPQATPVSKQQSQGSIGETTPAAGMWTLGTPAADVWILGTPAADVWTSMEAASGEGSAAGDLDAATGDRGPQATLSQTPAVGPWGPPGKESSVKRTFPEDESSSRTLAPVSTMLALFMLMALVLLQRKLWRRRTSQEAERVTLIQMTHFLEVNPQADQLPHVERKMLQDDSLPAGASLTAPERNPGP

SEQ ID NO: 29 - protein, 287 aa, Homo Sapiens
MDPKQTTLLCLVLCLGQRIQAQEGDFPMPFISAKSSPVIPLDGSVKIQCQAIREAYLTQLMIIKNSTYREIGRRLKFWNETDPEFVIDHMDANKAGRYQCQYRIGHYRFRYSDTLELVVTGLYGKPFLSADRGLVLMPGENISLTCSSAHIPFDRFSLAKEGELSLPQHQSGEHPANFSLGPVDLNVSGIYRCYGWYNRSPYLWSFPSNALELVVTDSIHQDYTTQNLIRMAVAGLVLVALLAILVENWHSHTALNKEASADVAEPSWSQQMCQPGLTFARTPSVCK

SEQ ID NO: 30 - protein, 86 aa, Homo Sapiens MAPAMESPTLLCVALLFFAPDGVLAVPQKPKVSLNPPWNRIFKGENVTLTCNGNNFFEVS STKWFHNGSLSEETNSSLNIVNAKFEDSGEYKCQHQQVNESEPVYLEVFSDWLLLQASAE VVMEGQPLFLRCHGWRNWDVYKVIYYKDGEALKYWYENHNISITNATVEDSGTYYCTGKV WQLDYESEPLNITVIKAPREKYWLQFFIPLLVVILFAVDTGLFISTQQQVTFLLKIKRTR KGFRLLNPHPKPNPKNN <FCERG;Protein/1;Homo Sapiens
MIPAVVLLLLLLVEQAAALGEPQLCYILDAILFLYGIVLTLLYCRLKIQVRKAAITSYEKSDGVYTGLSTRNQETYETLKHEKPPQ

SEQ ID NO: 31 - protein, 374 aa, Homo Sapiens
MWFLTTLLLWVPVDGQVDTTKAVITLQPPWVSVFQEETVTLHCEVLHLPGSSSTQWFLNGTATQTSTPSYRITSASVNDSGEYRCQRGLSGRSDPIQLEIHRGWLLLQVSSRVFTEGEPLALRCHAWKDKLVYNVLYYRNGKAFKFFHWNSNLTILKTNISHNGTYHCSGMGKHRYTSAGISVTVKELFPAPVLNASVTSPLLEGNLVTLSCETKLLLQRPGLQLYFSFYMGSKTLRGRNTSSEYQILTARREDSGLYWCEAATEDGNVLKRSPELELQVLGLQLPTPVWFHVLFYLAVGIMFLVNTVLWVTIRKELKRKKKWDLEISLDSGHEKKVISSLQEDRHLEEELKCQEQKEEQLQEGVHRKEPQGAT

SEQ ID NO: 32 - protein, 280 aa, Homo Sapiens
MWFLTTLLLWVPVDGQVDTTKAVITLQPPWVSVFQEETVTLHCEVLHLPGSSSTQWFLNGTATQTSTPSYRITSASVNDSGEYRCQRGLSGRSDPIQLEIHRGWLLLQVSSRVFMEGEPLALRCHAWKDKLVYNVLYYRNGKAFKFFHWNSNLTILKTNISHNGTYHCSGMGKHRYTSAGISQYTVKGLQLPTPVWFHVLFYLAVGIMFLVNTVLWVTIRKELKRKKKWNLEISLDSGHEKKVISSLQEDRHLEEELKCQEQKEEQLQEGVHRKEPQGAT

SEQ ID NO: 33 - protein, 416 aa, Artificial sequence
  Artificial sequence comprising at least one exosomal polypeptide and at least one Fc binding polypeptide
MGLSTVPDLLLPLVLLELLVGIYPSGVIGLVPHLGDREKRDSVCPQGKYIHPQNNSICCTKCHKGTYLYNDCPGPGQDTDCRECESGSFTASENHLRHCLSCSKCRKEMGQVEISSCTVDRDTVCGCRKNQYRHYWSENLFQCFNCSLCLNGTVHLSCQEKQNTVCTCHAGFFLRENECVSCSNCKKSLECTKLCLNGGGGSGGGGSGRDNKFNKEQQNAFYEILHLPNLNEEQRNAFIQSLKDDPSQSANLLAEAKKLNDAQAPKPQGTEDSGTTVLLPLVIFFGLCLLSLLFIGLMYRYQRWKGTNGGGGSGRGYIPEAPRDGQAYVRKDGEWVFLSTFLSPANGGGGSGRSLYPSLEDLKVDKVIQAQTAFSANPANPAILSEASAPIPHDGNLYPRLYPELSQYMGLSLEGG

SEQ ID NO: 34 - protein, 836 aa, Artificial sequence
  Artificial sequence comprising at least one exosomal polypeptide and at least one Fc binding polypeptide
MSAPRIWLAQALLFFLTTESIGQLLEPCGYIYPEFPVVQRGSNFTAICVLKEACLQHYYVNASYIVWKTNHAAVPREQVTVINRTTSSVTFTDVVLPSVQLTCNILSFGQIEQNVYGVTMLSGFPPDKPTNLTCIVNEGKNMLCQWDPGRETYLETNYTLKSEWATEKFPDCQSKHGTSCMVSYMPTYYVNIEVWVEAENALGKVSSESINFDPVDKVKPTPPYNLSVTNSEELSSILKLSWVSSGLGGLLDLKSDIQYRTKDASTWIQVPLEDTMSPRTSFTVQDLKPFTEYVFRIRSIKDSGKGYWSDWSEEASGTTYEDRPSRPPSFWYKTNPSHGQEYRSVRLIWKALPLSEANGKILDYEVILTQSKSVSQTYTVTGTELTVNLTNDRYVASLAARNKVGKSAAAVLTIPSPHVTAGSGSGSGSGSRMKQKKLVGERGSGSGSGSGSDNKFNKEQQNAFYEILHLPNLNEEQRNAFIQSLKDDPSQSANLLAEAKKLNDAQAPKAAPARGPTVRTKKVGKNEAVLAWDQIPVDDQNGFIRNYSISYRTSVGKEMVVHVDSSHTEYTLSSLSSDTLYMVRMAAYTDEGGKDGPEFTFTTPKFAQGEIEAIVVPVCLAFLLTTLLGVLFCFNKRDLIKKHIWPNVPDPSKSHIAQWSPHTPPRHNFNSKDQGSGSGSGSGSRMKQLEDKVEELLSKNYHLENEVARLKKLVGERGSGSGSGSGSSLYPSLEDLKVDKVIQAQTAYSANPASQAFVLVDASAALPPDGNLYPKLYPELSQYMGLSLNEAEICESMPMVSGAPAQGQLVARPSSVNYMVAPVTGNDAGIRRAEIK

SEQ ID NO: 35 - protein, 359 aa, Artificial sequence
  Artificial sequence comprising at least one exosomal polypeptide and at least one Fc binding polypeptide
AVEGGMKCVKFLLYVLLLAFCACAVGLIAVGVGAQLVLSQTGTDNKFNKEQQNAFYEILHLPNLNEEQRNAFIQSLKDDPSQSANLLAEAKKLNDAQAPKGTIIQGATPGSLLPVVIIAVGVFLFLVAFVGCCGACKENYCLMITFAIFLSLIMLVEVAAAIAGYVFRDKVMSEFNNNFRQQMENYPKNNHTASILDRMQADFKCCGAGSDNKFNKEQQNAFYEILHLPNLNEEQRNAFIQSLKDDPSQSANLLAEAKKLNDAQAPKGSANYTDWEKIPSMSKNRVPDSCCINVTVGCGINFNEKAIHKEGCVEKIGGWLRKNVLVVAAAALGIAFVEVLGIVFACCLVKSIRSGYEVM

SEQ ID NO: 36 - protein, 532 aa, Artificial sequence
  Artificial sequence comprising at least one exosomal polypeptide and at least one Fc binding polypeptide
MDNKFNKEQQNAFYEILHLPNLNEEQRNAFIQSLKDDPSQSANLLAEAKKLNDAQAPKGSGSGGSGSGSVCFRLFPVPGSGLVLVCLVLGAVRSYAKSSVGRQGSGSGSGLELNLTDSENATCLYAKWQMNFTVRYETTNKTYKTVTISDHGTVTYNGSICGDDQNGPKIAVQFGPGFSWIANFTKAASTYSIDSVSFSYNTGDNTTFPDAEDKGILTVDELLAIRIPLNDLFRCNSLSTLEKNDVVQHYWDVLVQAFVQNGTVSTNEFLCDKDKTSTVAPTIHTTVPSPTTTPTPKEKPEAGTYSVNNGNDTCLLATMGLQLNITQDKVASVININPNTTHSTGSCRSHTALLRLNSSTIKYLDFVFAVKNENRFYLKEVNISMYLVNGSVFSIANNNLSYWDAPLGSSYMCNKEQTVSVSGAFQINTFDLRVQPFNVTQGKYSTAQDCSADDDNFLVPIAVGAALAGVLILVLLAYFIGLKHHHAGYEQFGSGSGSGSGSGSTGGSRTGSGSGSGSGSGSPGHHHHHHHH

SEQ ID NO: 37 - protein, 514 aa, Artificial sequence
  Artificial sequence comprising at least one exosomal polypeptide and at least one Fc binding polypeptide
MVCFRLFPVPGSGLVLVCLVLGAVRSYAKSSVGRQDNKFNKEQQNAFYEILHLPNLNEEQRNAFIQSLKDDPSQSANLLAEAKKLNDAQAPKGGGGSGGGGSLELNLTDSENATCLYAKWQMNFTVRYETTNKTYKTVTISDHGTVTYNGSICGDDQNGPKIAVQFGPGFSWIANFTKAASTYSIDSVSFSYNTGDNTTFPDAEDKGILTVDELLAIRIPLNDLFRCNSLSTLEKNDVVQHYWDVLVQAFVQNGTVSTNEFLCDKDKTSTVAPTIHTTVPSPTTTPTPKEKPEAGTYSVNNGNDTCLLATMGLQLNITQDKVASVININPNTTHSTGSCRSHTALLRLNSSTIKYLDFVFAVKNENRFYLKEVNISMYLVNGSVFSIANNNLSYWDAPLGSSYMCNKEQTVSVSGAFQINTFDLRVQPFNVTQGKYSTAQDCSADDDNFLVPIAVGAALAGVLILVLLAYFIGLKHHHAGYEQFGSGSGSGSGSGSTGGSRTGSGSGSGSGSGS

SEQ ID NO: 38 - protein, 826 aa, Artificial sequence
  Artificial sequence comprising at least one exosomal polypeptide and at least one Fc binding polypeptide
MDQARSAFSNLFGGEPLSYTRFSLARQVDGDNSHVEMKLAVDEEENADNNTKANVTKPKRCSGSICYGTIAVIVFFLIGFMIGYLGYCKGVEPKTECERLAGTESPVREEPGEDFPAARRLYWDDLKRKLSEKLDSTDFTGTIKLLNENSYVPREAGSQKDENLALYVENQFREFKLSKVWRDQHFVKIQVKDSAQNSVIIVDKNGRLVYLVENPGGYVAYSKAATVTGKLVHANFGTKKDFEDLYTPVNGSIVIVRAGKITFAEKVANAESLNAIGVLIYMDQTKFPIVNAELSFFGHAHLGTGDPYTPGFPSFNHTQFPPSRSSGLPNIPVQTISRAAAEKLFGNMEGDCPSDWKTDSTCRMVTSESKNVKLTVSNVLKEIKILNIFGVIKGFVEPDHYVVVGAQRDAWGPGAAKSGVGTALLLKLAQMFSDMVLKDGFQPSRSIIFASWSAGDFGSVGATEWLEGYLSSLHLKAFTYINLDKAVLGTSNFKVSASPLLYTLIEKTMQNVKHPVTGQFLYQDSNWASKVEKLTLDNAAFPFLAYSGIPAVSFCFCEDTDYPYLGTTMDTYKELIERIPELNKVARAAAEVAGQFVIKLTHDVELNLDYERYNSQLLSFVRDLNQYRADIKEMGLSLQWLYSARGDFFRATSRLTTDFGNAEKTDRFVMKKLNDRVMRVEYHFLSPYVSPKESPFRHVFWGSGSHTLPALLENLKLRKQNNGAFNETLFRNQLALATWTIQGAANALSGDVWDIDNEFGGGGSGGGGSDNKFNKEQQNAFYEILHLPNLNEEQRNAFIQSLKDDPSQSANLLAEAKKLNDAQAPK

SEQ ID NO: 39 - protein, 726 aa, Artificial sequence
  Artificial sequence comprising at least one exosomal polypeptide and at least one Fc binding polypeptide
MAESHLSLLYHLTAVSSPAPGTPAFWVSGWLGPQQYLSYNSLRGEAEPCGAWVWENQVSWYWEKETTDLRIKEKLFLEAFKALGGKGPYTLQGLLGCELGPDNTSVPTAKFALNGEEFMNFDLKQGTWGGDWPEALAISQRWQQQDKAANKELTFLLFSCPHRLREHLERGRGNLEWKEPPSMRLKARPSSPGFSVLTCSAFSFYPPELQLRFLRNGLAAGTGQGDFGPNSDGSFHASSSLTVKSGDEHHYCGSGSGGSGSGSVCFRLFPVPGSGLVLVCLVLGAVRSYAKSSVGRQGSGSGSGLELNLTDSENATCLYAKWQMNFTVRYETTNKTYKTVTISDHGTVTYNGSICGDDQNGPKIAVQFGPGFSWIANFTKAASTYSIDSVSFSYNTGDNTTFPDAEDKGILTVDELLAIRIPLNDLFRCNSLSTLEKNDVVQHYWDVLVQAFVQNGTVSTNEFLCDKDKTSTVAPTIHTTVPSPTTTPTPKEKPEAGTYSVNNGNDTCLLATMGLQLNITQDKVASVININPNTTHSTGSCRSHTALLRLNSSTIKYLDFVFAVKNENRFYLKEVNISMYLVNGSVFSIANNNLSYWDAPLGSSYMCNKEQTVSVSGAFQINTFDLRVQPFNVTQGKYSTAQDCSADDDNFLVPIAVGAALAGVLILVLLAYFIGLKHHHAGYEQFGSGSGSGSGSGSTGGSRTGSGSGSGSGSGSPGHHHHHHHH

SEQ ID NO: 40 - protein, 710 aa, Artificial sequence
  Artificial sequence comprising at least one exosomal polypeptide and at least one Fc binding polypeptide
MVCFRLFPVPGSGLVLVCLVLGAVRSYAKSSVGRQAESHLSLLYHLTAVSSPAPGTPAFWVSGWLGPQQYLSYNSLRGEAEPCGAWVWENQVSWYWEKETTDLRIKEKLFLEAFKALGGKGPYTLQGLLGCELGPDNTSVPTAKFALNGEEFMNFDLKQGTWGGDWPEALAISQRWQQQDKAANKELTFLLFSCPHRLREHLERGRGNLEWKEPPSMRLKARPSSPGFSVLTCSAFSFYPPELQLRFLRNGLAAGTGQGDFGPNSDGSFHASSSLTVKSGDEHHYCGGGGSGGGGSLELNLTDSENATCLYAKWQMNFTVRYETTNKTYKTVTISDHGTVTYNGSICGDDQNGPKIAVQFGPGFSWIANFTKAASTYSIDSVSFSYNTGDNTTFPDAEDKGILTVDELLAIRIPLNDLFRCNSLSTLEKNDVVQHYWDVLVQAFVQNGTVSTNEFLCDKDKTSTVAPTIHTTVPSPTTTPTPKEKPEAGTYSVNNGNDTCLLATMGLQLNITQDKVASVININPNTTHSTGSCRSHTALLRLNSSTIKYLDFVFAVKNENRFYLKEVNISMYLVNGSVFSIANNNLSYWDAPLGSSYMCNKEQTVSVSGAFQINTFDLRVQPFNVTQGKYSTAQDCSADDDNFLVPIAVGAALAGVLILVLLAYFIGLKHHHAGYEQFGSGSGSGSGSGSTGGSRTGSGSGSGSGSGSPG

SEQ ID NO: 41 - protein, 1020 aa, Artificial sequence
  Artificial sequence comprising at least one exosomal polypeptide and at least one Fc binding polypeptide
MDQARSAFSNLFGGEPLSYTRFSLARQVDGDNSHVEMKLAVDEEENADNNTKANVTKPKRCSGSICYGTIAVIVFFLIGFMIGYLGYCKGVEPKTECERLAGTESPVREEPGEDFPAARRLYWDDLKRKLSEKLDSTDFTGTIKLLNENSYVPREAGSQKDENLALYVENQFREFKLSKVWRDQHFVKIQVKDSAQNSVIIVDKNGRLVYLVENPGGYVAYSKAATVTGKLVHANFGTKKDFEDLYTPVNGSIVIVRAGKITFAEKVANAESLNAIGVLIYMDQTKFPIVNAELSFFGHAHLGTGDPYTPGFPSFNHTQFPPSRSSGLPNIPVQTISRAAAEKLFGNMEGDCPSDWKTDSTCRMVTSESKNVKLTVSNVLKEIKILNIFGVIKGFVEPDHYVVVGAQRDAWGPGAAKSGVGTALLLKLAQMFSDMVLKDGFQPSRSIIFASWSAGDFGSVGATEWLEGYLSSLHLKAFTYINLDKAVLGTSNFKVSASPLLYTLIEKTMQNVKHPVTGQFLYQDSNWASKVEKLTLDNAAFPFLAYSGIPAVSFCFCEDTDYPYLGTTMDTYKELIERIPELNKVARAAAEVAGQFVIKLTHDVELNLDYERYNSQLLSFVRDLNQYRADIKEMGLSLQWLYSARGDFFRATSRLTTDFGNAEKTDRFVMKKLNDRVMRVEYHFLSPYVSPKESPFRHVFWGSGSHTLPALLENLKLRKQNNGAFNETLFRNQLALATWTIQGAANALSGDVWDIDNEFGGGGSGGGGSAESHLSLLYHLTAVSSPAPGTPAFWVSGWLGPQQYLSYNSLRGEAEPCGAWVWENQVSWYWEKETTDLRIKEKLFLEAFKALGGKGPYTLQGLLGCELGPDNTSVPTAKFALNGEEFMNFDLKQGTWGGDWPEALAISQRWQQQDKAANKELTFLLFSCPHRLREHLERGRGNLEWKEPPSMRLKARPSSPGFSVLTCSAFSFYPPELQLRFLRNGLAAGTGQGDFGPNSDGSFHASSSLTVKSGDEHHYC

SEQ ID NO: 42 - protein, 610 aa, Artificial sequence
  Artificial sequence comprising at least one exosomal polypeptide and at least one Fc binding polypeptide
MGLSTVPDLLLPLVLLELLVGIYPSGVIGLVPHLGDREKRDSVCPQGKYIHPQNNSICCTKCHKGTYLYNDCPGPGQDTDCRECESGSFTASENHLRHCLSCSKCRKEMGQVEISSCTVDRDTVCGCRKNQYRHYWSENLFQCFNCSLCLNGTVHLSCQEKQNTVCTCHAGFFLRENECVSCSNCKKSLECTKLCLNGGGGSGGGGSGRAESHLSLLYHLTAVSSPAPGTPAFWVSGWLGPQQYLSYNSLRGEAEPCGAWVWENQVSWYWEKETTDLRIKEKLFLEAFKALGGKGPYTLQGLLGCELGPDNTSVPTAKFALNGEEFMNFDLKQGTWGGDWPEALAISQRWQQQDKAANKELTFLLFSCPHRLREHLERGRGNLEWKEPPSMRLKARPSSPGFSVLTCSAFSFYPPELQLRFLRNGLAAGTGQGDFGPNSDGSFHASSSLTVKSGDEHHYCPQGTEDSGTTVLLPLVIFFGLCLLSLLFIGLMYRYQRWKGTNGGGGSGRGYIPEAPRDGQAYVRKDGEWVFLSTFLSPANGGGGSGRSLYPSLEDLKVDKVIQAQTAFSANPANPAILSEASAPIPHDGNLYPRLYPELSQYMGLSLEGG

SEQ ID NO: 43 - protein, 1030 aa, Artificial sequence
  Artificial sequence comprising at least one exosomal polypeptide and at least one Fc binding polypeptide
MSAPRIWLAQALLFFLTTESIGQLLEPCGYIYPEFPVVQRGSNFTAICVLKEACLQHYYVNASYIVWKTNHAAVPREQVTVINRTTSSVTFTDVVLPSVQLTCNILSFGQIEQNVYGVTMLSGFPPDKPTNLTCIVNEGKNMLCQWDPGRETYLETNYTLKSEWATEKFPDCQSKHGTSCMVSYMPTYYVNIEVWVEAENALGKVSSESINFDPVDKVKPTPPYNLSVTNSEELSSILKLSWVSSGLGGLLDLKSDIQYRTKDASTWIQVPLEDTMSPRTSFTVQDLKPFTEYVFRIRSIKDSGKGYWSDWSEEASGTTYEDRPSRPPSFWYKTNPSHGQEYRSVRLIWKALPLSEANGKILDYEVILTQSKSVSQTYTVTGTELTVNLTNDRYVASLAARNKVGKSAAAVLTIPSPHVTAGSGSGSGSGSRMKQKKLVGERGSGSGSGSGSAESHLSLLYHLTAVSSPAPGTPAFWVSGWLGPQQYLSYNSLRGEAEPCGAWVWENQVSWYWEKETTDLRIKEKLFLEAFKALGGKGPYTLQGLLGCELGPDNTSVPTAKFALNGEEFMNFDLKQGTWGGDWPEALAISQRWQQQDKAANKELTFLLFSCPHRLREHLERGRGNLEWKEPPSMRLKARPSSPGFSVLTCSAFSFYPPELQLRFLRNGLAAGTGQGDFGPNSDGSFHASSSLTVKSGDEHHYCAAPARGPTVRTKKVGKNEAVLAWDQIPVDDQNGFIRNYSISYRTSVGKEMVVHVDSSHTEYTLSSLSSDTLYMVRMAAYTDEGGKDGPEFTFTTPKFAQGEIEAIVVPVCLAFLLTTLLGVLFCFNKRDLIKKHIWPNVPDPSKSHIAQWSPHTPPRHNFNSKDQGSGSGSGSGSRMKQLEDKVEELLSKNYHLENEVARLKKLVGERGSGSGSGSGSSLYPSLEDLKVDKVIQAQTAYSANPASQAFVLVDASAALPPDGNLYPKLYPELSQYMGLSLNEAEICESMPMVSGAPAQGQLVARPSSVNYMVAPVTGNDAGIRRAEIK

SEQ ID NO: 44 - protein, 747 aa, Artificial sequence
  Artificial sequence comprising at least one exosomal polypeptide and at least one Fc binding polypeptide
AVEGGMKCVKFLLYVLLLAFCACAVGLIAVGVGAQLVLSQTGTAESHLSLLYHLTAVSSPAPGTPAFWVSGWLGPQQYLSYNSLRGEAEPCGAWVWENQVSWYWEKETTDLRIKEKLFLEAFKALGGKGPYTLQGLLGCELGPDNTSVPTAKFALNGEEFMNFDLKQGTWGGDWPEALAISQRWQQQDKAANKELTFLLFSCPHRLREHLERGRGNLEWKEPPSMRLKARPSSPGFSVLTCSAFSFYPPELQLRFLRNGLAAGTGQGDFGPNSDGSFHASSSLTVKSGDEHHYCGTIIQGATPGSLLPVVIIAVGVFLFLVAFVGCCGACKENYCLMITFAIFLSLIMLVEVAAAIAGYVFRDKVMSEFNNNFRQQMENYPKNNHTASILDRMQADFKCCGAGSAESHLSLLYHLTAVSSPAPGTPAFWVSGWLGPQQYLSYNSLRGEAEPCGAWVWENQVSWYWEKETTDLRIKEKLFLEAFKALGGKGPYTLQGLLGCELGPDNTSVPTAKFALNGEEFMNFDLKQGTWGGDWPEALAISQRWQQQDKAANKELTFLLFSCPHRLREHLERGRGNLEWKEPPSMRLKARPSSPGFSVLTCSAFSFYPPELQLRFLRNGLAAGTGQGDFGPNSDGSFHASSSLTVKSGDEHHYCGSANYTDWEKIPSMSKNRVPDSCCINVTVGCGINFNEKAIHKEGCVEKIGGWLRKNVLVVAAAALGIAFVEVLGIVFACCLVKSIRSGYEVM

SEQ ID NO: 45 - protein, 610 aa, Artificial sequence
  Artificial sequence comprising at least one exosomal polypeptide and at least one Fc binding polypeptide
MGLSTVPDLLLPLVLLELLVGIYPSGVIGLVPHLGDREKRDSVCPQGKYIHPQNNSICCTKCHKGTYLYNDCPGPGQDTDCRECESGSFTASENHLRHCLSCSKCRKEMGQVEISSCTVDRDTVCGCRKNQYRHYWSENLFQCFNCSLCLNGTVHLSCQEKQNTVCTCHAGFFLRENECVSCSNCKKSLECTKLCLNGGGGSGGGGSGRQVDTTKAVITLQPPWVSVFQEETVTLHCEVLHLPGSSSTQWFLNGTATQTSTPSYRITSASVNDSGEYRCQRGLSGRSDPIQLEIHRGWLLLQVSSRVFTEGEPLALRCHAWKDKLVYNVLYYRNGKAFKFFHWNSNLTILKTNISHNGTYHCSGMGKHRYTSAGISVTVKELFPAPVLNASVTSPLLEGNLVTLSCETKLLLQRPGLQLYFSFYMGSKTLRGRNTSSEYQILTARREDSGLYWCEAATEDPQGTEDSGTTVLLPLVIFFGLCLLSLLFIGLMYRYQRWKGTNGGGGSGRGYIPEAPRDGQAYVRKDGEWVFLSTFLSPANGGGGSGRSLYPSLEDLKVDKVIQAQTAFSANPANPAILSEASAPIPHDGNLYPRLYPELSQYMGLSLEGG

SEQ ID NO: 46 - protein, 1030 aa, Artificial sequence
  Artificial sequence comprising at least one exosomal polypeptide and at least one Fc binding polypeptide
MSAPRIWLAQALLFFLTTESIGQLLEPCGYIYPEFPVVQRGSNFTAICVLKEACLQHYYVNASYIVWKTNHAAVPREQVTVINRTTSSVTFTDVVLPSVQLTCNILSFGQIEQNVYGVTMLSGFPPDKPTNLTCIVNEGKNMLCQWDPGRETYLETNYTLKSEWATEKFPDCQSKHGTSCMVSYMPTYYVNIEVWVEAENALGKVSSESINFDPVDKVKPTPPYNLSVTNSEELSSILKLSWVSSGLGGLLDLKSDIQYRTKDASTWIQVPLEDTMSPRTSFTVQDLKPFTEYVFRIRSIKDSGKGYWSDWSEEASGTTYEDRPSRPPSFWYKTNPSHGQEYRSVRLIWKALPLSEANGKILDYEVILTQSKSVSQTYTVTGTELTVNLTNDRYVASLAARNKVGKSAAAVLTIPSPHVTAGSGSGSGSGSRMKQKKLVGERGSGSGSGSGSQVDTTKAVITLQPPWVSVFQEETVTLHCEVLHLPGSSSTQWFLNGTATQTSTPSYRITSASVNDSGEYRCQRGLSGRSDPIQLEIHRGWLLLQVSSRVFTEGEPLALRCHAWKDKLVYNVLYYRNGKAFKFFHWNSNLTILKTNISHNGTYHCSGMGKHRYTSAGISVTVKELFPAPVLNASVTSPLLEGNLVTLSCETKLLLQRPGLQLYFSFYMGSKTLRGRNTSSEYQILTARREDSGLYWCEAATEDAAPARGPTVRTKKVGKNEAVLAWDQIPVDDQNGFIRNYSISYRTSVGKEMVVHVDSSHTEYTLSSLSSDTLYMVRMAAYTDEGGKDGPEFTFTTPKFAQGEIEAIVVPVCLAFLLTTLLGVLFCFNKRDLIKKHIWPNVPDPSKSHIAQWSPHTPPRHNFNSKDQGSGSGSGSGSRMKQLEDKVEELLSKNYHLENEVARLKKLVGERGSGSGSGSGSSLYPSLEDLKVDKVIQAQTAYSANPASQAFVLVDASAALPPDGNLYPKLYPELSQYMGLSLNEAEICESMPMVSGAPAQGQLVARPSSVNYMVAPVTGNDAGIRRAEIK

SEQ ID NO: 47 - protein, 747 aa, Artificial sequence
  Artificial sequence comprising at least one exosomal polypeptide and at least one Fc binding polypeptide
AVEGGMKCVKFLLYVLLLAFCACAVGLIAVGVGAQLVLSQTGTQVDTTKAVITLQPPWVSVFQEETVTLHCEVLHLPGSSSTQWFLNGTATQTSTPSYRITSASVNDSGEYRCQRGLSGRSDPIQLEIHRGWLLLQVSSRVFTEGEPLALRCHAWKDKLVYNVLYYRNGKAFKFFHWNSNLTILKTNISHNGTYHCSGMGKHRYTSAGISVTVKELFPAPVLNASVTSPLLEGNLVTLSCETKLLLQRPGLQLYFSFYMGSKTLRGRNTSSEYQILTARREDSGLYWCEAATEDGTIIQGATPGSLLPVVIIAVGVFLFLVAFVGCCGACKENYCLMITFAIFLSLIMLVEVAAAIAGYVFRDKVMSEFNNNFRQQMENYPKNNHTASILDRMQADFKCCGAGSQVDTTKAVITLQPPWVSVFQEETVTLHCEVLHLPGSSSTQWFLNGTATQTSTPSYRITSASVNDSGEYRCQRGLSGRSDPIQLEIHRGWLLLQVSSRVFTEGEPLALRCHAWKDKLVYNVLYYRNGKAFKFFHWNSNLTILKTNISHNGTYHCSGMGKHRYTSAGISVTVKELFPAPVLNASVTSPLLEGNLVTLSCETKLLLQRPGLQLYFSFYMGSKTLRGRNTSSEYQILTARREDSGLYWCEAATEDGSANYTDWEKIPSMSKNRVPDSCCINVTVGCGINFNEKAIHKEGCVEKIGGWLRKNVLVVAAAALGIAFVEVLGIVFACCLVKSIRSGYEVM

SEQ ID NO: 48 - protein, 726 aa, Artificial sequence
  Artificial sequence comprising at least one exosomal polypeptide and at least one Fc binding polypeptide
MQVDTTKAVITLQPPWVSVFQEETVTLHCEVLHLPGSSSTQWFLNGTATQTSTPSYRITSASVNDSGEYRCQRGLSGRSDPIQLEIHRGWLLLQVSSRVFTEGEPLALRCHAWKDKLVYNVLYYRNGKAFKFFHWNSNLTILKTNISHNGTYHCSGMGKHRYTSAGISVTVKELFPAPVLNASVTSPLLEGNLVTLSCETKLLLQRPGLQLYFSFYMGSKTLRGRNTSSEYQILTARREDSGLYWCEAATEDGSGSGGSGSGSVCFRLFPVPGSGLVLVCLVLGAVRSYAKSSVGRQGSGSGSGLELNLTDSENATCLYAKWQMNFTVRYETTNKTYKTVTISDHGTVTYNGSICGDDQNGPKIAVQFGPGFSWIANFTKAASTYSIDSVSFSYNTGDNTTFPDAEDKGILTVDELLAIRIPLNDLFRCNSLSTLEKNDVVQHYWDVLVQAFVQNGTVSTNEFLCDKDKTSTVAPTIHTTVPSPTTTPTPKEKPEAGTYSVNNGNDTCLLATMGLQLNITQDKVASVININPNTTHSTGSCRSHTALLRLNSSTIKYLDFVFAVKNENRFYLKEVNISMYLVNGSVFSIANNNLSYWDAPLGSSYMCNKEQTVSVSGAFQINTFDLRVQPFNVTQGKYSTAQDCSADDDNFLVPIAVGAALAGVLILVLLAYFIGLKHHHAGYEQFGSGSGSGSGSGSTGGSRTGSGSGSGSGSGSPGHHHHHHHH

SEQ ID NO: 49 - protein, 710 aa, Artificial sequence
  Artificial sequence comprising at least one exosomal polypeptide and at least one Fc binding polypeptide
MVCFRLFPVPGSGLVLVCLVLGAVRSYAKSSVGRQQVDTTKAVITLQPPWVSVFQEETVTLHCEVLHLPGSSSTQWFLNGTATQTSTPSYRITSASVNDSGEYRCQRGLSGRSDPIQLEIHRGWLLLQVSSRVFTEGEPLALRCHAWKDKLVYNVLYYRNGKAFKFFHWNSNLTILKTNISHNGTYHCSGMGKHRYTSAGISVTVKELFPAPVLNASVTSPLLEGNLVTLSCETKLLLQRPGLQLYFSFYMGSKTLRGRNTSSEYQILTARREDSGLYWCEAATEDGGGGSGGGGSLELNLTDSENATCLYAKWQMNFTVRYETTNKTYKTVTISDHGTVTYNGSICGDDQNGPKIAVQFGPGFSWIANFTKAASTYSIDSVSFSYNTGDNTTFPDAEDKGILTVDELLAIRIPLNDLFRCNSLSTLEKNDVVQHYWDVLVQAFVQNGTVSTNEFLCDKDKTSTVAPTIHTTVPSPTTTPTPKEKPEAGTYSVNNGNDTCLLATMGLQLNITQDKVASVININPNTTHSTGSCRSHTALLRLNSSTIKYLDFVFAVKNENRFYLKEVNISMYLVNGSVFSIANNNLSYWDAPLGSSYMCNKEQTVSVSGAFQINTFDLRVQPFNVTQGKYSTAQDCSADDDNFLVPIAVGAALAGVLILVLLAYFIGLKHHHAGYEQFGSGSGSGSGSGSTGGSRTGSGSGSGSGSGSPG

SEQ ID NO: 50 - protein, 1020 aa, Artificial sequence
  Artificial sequence comprising at least one exosomal polypeptide and at least one Fc binding polypeptide
MDQARSAFSNLFGGEPLSYTRFSLARQVDGDNSHVEMKLAVDEEENADNNTKANVTKPKRCSGSICYGTIAVIVFFLIGFMIGYLGYCKGVEPKTECERLAGTESPVREEPGEDFPAARRLYWDDLKRKLSEKLDSTDFTGTIKLLNENSYVPREAGSQKDENLALYVENQFREFKLSKVWRDQHFVKIQVKDSAQNSVIIVDKNGRLVYLVENPGGYVAYSKAATVTGKLVHANFGTKKDFEDLYTPVNGSIVIVRAGKITFAEKVANAESLNAIGVLIYMDQTKFPIVNAELSFFGHAHLGTGDPYTPGFPSFNHTQFPPSRSSGLPNIPVQTISRAAAEKLFGNMEGDCPSDWKTDSTCRMVTSESKNVKLTVSNVLKEIKILNIFGVIKGFVEPDHYVVVGAQRDAWGPGAAKSGVGTALLLKLAQMFSDMVLKDGFQPSRSIIFASWSAGDFGSVGATEWLEGYLSSLHLKAFTYINLDKAVLGTSNFKVSASPLLYTLIEKTMQNVKHPVTGQFLYQDSNWASKVEKLTLDNAAFPFLAYSGIPAVSFCFCEDTDYPYLGTTMDTYKELIERIPELNKVARAAAEVAGQFVIKLTHDVELNLDYERYNSQLLSFVRDLNQYRADIKEMGLSLQWLYSARGDFFRATSRLTTDFGNAEKTDRFVMKKLNDRVMRVEYHFLSPYVSPKESPFRHVFWGSGSHTLPALLENLKLRKQNNGAFNETLFRNQLALATWTIQGAANALSGDVWDIDNEFGGGGSGGGGSQVDTTKAVITLQPPWVSVFQEETVTLHCEVLHLPGSSSTQWFLNGTATQTSTPSYRITSASVNDSGEYRCQRGLSGRSDPIQLEIHRGWLLLQVSSRVFTEGEPLALRCHAWKDKLVYNVLYYRNGKAFKFFHWNSNLTILKTNISHNGTYHCSGMGKHRYTSAGISVTVKELFPAPVLNASVTSPLLEGNLVTLSCETKLLLQRPGLQLYFSFYMGSKTLRGRNTSSEYQILTARREDSGLYWCEAATED

SEQ ID NO: 51 - protein, 565 aa, Artificial sequence
  Artificial sequence comprising at least one exosomal polypeptide and at least one Fc binding polypeptide
MGLSTVPDLLLPLVLLELLVGIYPSGVIGLVPHLGDREKRDSVCPQGKYIHPQNNSICCTKCHKGTYLYNDCPGPGQDTDCRECESGSFTASENHLRHCLSCSKCRKEMGQVEISSCTVDRDTVCGCRKNQYRHYWSENLFQCFNCSLCLNGTVHLSCQEKQNTVCTCHAGFFLRENECVSCSNCKKSLECTKLCLNGGGGSGGGGSGRQEGDFPMPFISAKSSPVIPLDGSVKIQCQAIREAYLTQLMIIKNSTYREIGRRLKFWNETDPEFVIDHMDANKAGRYQCQYRIGHYRFRYSDTLELVVTGLYGKPFLSADRGLVLMPGENISLTCSSAHIPFDRFSLAKEGELSLPQHQSGEHPANFSLGPVDLNVSGIYRCYGWYNRSPYLWSFPSNALELVVTDSIHQDYTTQNPQGTEDSGTTVLLPLVIFFGLCLLSLLFIGLMYRYQRWKGTNGGGGSGRGYIPEAPRDGQAYVRKDGEWVFLSTFLSPANGGGGSGRSLYPSLEDLKVDKVIQAQTAFSANPANPAILSEASAPIPHDGNLYPRLYPELSQYMGLSLEGG

SEQ ID NO: 52 - protein, 985 aa, Artificial sequence
  Artificial sequence comprising at least one exosomal polypeptide and at least one Fc binding polypeptide
MSAPRIWLAQALLFFLTTESIGQLLEPCGYIYPEFPVVQRGSNFTAICVLKEACLQHYYVNASYIVWKTNHAAVPREQVTVINRTTSSVTFTDVVLPSVQLTCNILSFGQIEQNVYGVTMLSGFPPDKPTNLTCIVNEGKNMLCQWDPGRETYLETNYTLKSEWATEKFPDCQSKHGTSCMVSYMPTYYVNIEVWVEAENALGKVSSESINFDPVDKVKPTPPYNLSVTNSEELSSILKLSWVSSGLGGLLDLKSDIQYRTKDASTWIQVPLEDTMSPRTSFTVQDLKPFTEYVFRIRSIKDSGKGYWSDWSEEASGTTYEDRPSRPPSFWYKTNPSHGQEYRSVRLIWKALPLSEANGKILDYEVILTQSKSVSQTYTVTGTELTVNLTNDRYVASLAARNKVGKSAAAVLTIPSPHVTAGSGSGSGSGSRMKQKKLVGERGSGSGSGSGSQEGDFPMPFISAKSSPVIPLDGSVKIQCQAIREAYLTQLMIIKNSTYREIGRRLKFWNETDPEFVIDHMDANKAGRYQCQYRIGHYRFRYSDTLELVVTGLYGKPFLSADRGLVLMPGENISLTCSSAHIPFDRFSLAKEGELSLPQHQSGEHPANFSLGPVDLNVSGIYRCYGWYNRSPYLWSFPSNALELVVTDSIHQDYTTQNAAPARGPTVRTKKVGKNEAVLAWDQIPVDDQNGFIRNYSISYRTSVGKEMVVHVDSSHTEYTLSSLSSDTLYMVRMAAYTDEGGKDGPEFTFTTPKFAQGEIEAIVVPVCLAFLLTTLLGVLFCFNKRDLIKKHIWPNVPDPSKSHIAQWSPHTPPRHNFNSKDQGSGSGSGSGSRMKQLEDKVEELLSKNYHLENEVARLKKLVGERGSGSGSGSGSSLYPSLEDLKVDKVIQAQTAYSANPASQAFVLVDASAALPPDGNLYPKLYPELSQYMGLSLNEAEICESMPMVSGAPAQGQLVARPSSVNYMVAPVTGNDAGIRRAEIK

SEQ ID NO: 53 - protein, 657 aa, Artificial sequence
  Artificial sequence comprising at least one exosomal polypeptide and at least one Fc binding polypeptide
AVEGGMKCVKFLLYVLLLAFCACAVGLIAVGVGAQLVLSQTGTQEGDFPMPFISAKSSPVIPLDGSVKIQCQAIREAYLTQLMIIKNSTYREIGRRLKFWNETDPEFVIDHMDANKAGRYQCQYRIGHYRFRYSDTLELVVTGLYGKPFLSADRGLVLMPGENISLTCSSAHIPFDRFSLAKEGELSLPQHQSGEHPANFSLGPVDLNVSGIYRCYGWYNRSPYLWSFPSNALELVVTDSIHQDYTTQNGTIIQGATPGSLLPVVIIAVGVFLFLVAFVGCCGACKENYCLMITFAIFLSLIMLVEVAAAIAGYVFRDKVMSEFNNNFRQQMENYPKNNHTASILDRMQADFKCCGAGSQEGDFPMPFISAKSSPVIPLDGSVKIQCQAIREAYLTQLMIIKNSTYREIGRRLKFWNETDPEFVIDHMDANKAGRYQCQYRIGHYRFRYSDTLELVVTGLYGKPFLSADRGLVLMPGENISLTCSSAHIPFDRFSLAKEGELSLPQHQSGEHPANFSLGPVDLNVSGIYRCYGWYNRSPYLWSFPSNALELVVTDSIHQDYTTQNGSANYTDWEKIPSMSKNRVPDSCCINVTVGCGINFNEKAIHKEGCVEKIGGWLRKNVLVVAAAALGIAFVEVLGIVFACCLVKSIRSGYEVM

SEQ ID NO: 54 - protein, 681 aa, Artificial sequence
  Artificial sequence comprising at least one exosomal polypeptide and at least one Fc binding polypeptide
MQEGDFPMPFISAKSSPVIPLDGSVKIQCQAIREAYLTQLMIIKNSTYREIGRRLKFWNETDPEFVIDHMDANKAGRYQCQYRIGHYRFRYSDTLELVVTGLYGKPFLSADRGLVLMPGENISLTCSSAHIPFDRFSLAKEGELSLPQHQSGEHPANFSLGPVDLNVSGIYRCYGWYNRSPYLWSFPSNALELVVTDSIHQDYTTQNGSGSGGSGSGSVCFRLFPVPGSGLVLVCLVLGAVRSYAKSSVGRQGSGSGSGLELNLTDSENATCLYAKWQMNFTVRYETTNKTYKTVTISDHGTVTYNGSICGDDQNGPKIAVQFGPGFSWIANFTKAASTYSIDSVSFSYNTGDNTTFPDAEDKGILTVDELLAIRIPLNDLFRCNSLSTLEKNDVVQHYWDVLVQAFVQNGTVSTNEFLCDKDKTSTVAPTIHTTVPSPTTTPTPKEKPEAGTYSVNNGNDTCLLATMGLQLNITQDKVASVININPNTTHSTGSCRSHTALLRLNSSTIKYLDFVFAVKNENRFYLKEVNISMYLVNGSVFSIANNNLSYWDAPLGSSYMCNKEQTVSVSGAFQINTFDLRVQPFNVTQGKYSTAQDCSADDDNFLVPIAVGAALAGVLILVLLAYFIGLKHHHAGYEQFGSGSGSGSGSGSTGGSRTGSGSGSGSGSGSPGHHHHHHHH

SEQ ID NO: 55 - protein, 665 aa, Artificial sequence
  Artificial sequence comprising at least one exosomal polypeptide and at least one Fc binding polypeptide
MVCFRLFPVPGSGLVLVCLVLGAVRSYAKSSVGRQQEGDFPMPFISAKSSPVIPLDGSVKIQCQAIREAYLTQLMIIKNSTYREIGRRLKFWNETDPEFVIDHMDANKAGRYQCQYRIGHYRFRYSDTLELVVTGLYGKPFLSADRGLVLMPGENISLTCSSAHIPFDRFSLAKEGELSLPQHQSGEHPANFSLGPVDLNVSGIYRCYGWYNRSPYLWSFPSNALELVVTDSIHQDYTTQNGGGGSGGGGSLELNLTDSENATCLYAKWQMNFTVRYETTNKTYKTVTISDHGTVTYNGSICGDDQNGPKIAVQFGPGFSWIANFTKAASTYSIDSVSFSYNTGDNTTFPDAEDKGILTVDELLAIRIPLNDLFRCNSLSTLEKNDVVQHYWDVLVQAFVQNGTVSTNEFLCDKDKTSTVAPTIHTTVPSPTTTPTPKEKPEAGTYSVNNGNDTCLLATMGLQLNITQDKVASVININPNTTHSTGSCRSHTALLRLNSSTIKYLDFVFAVKNENRFYLKEVNISMYLVNGSVFSIANNNLSYWDAPLGSSYMCNKEQTVSVSGAFQINTFDLRVQPFNVTQGKYSTAQDCSADDDNFLVPIAVGAALAGVLILVLLAYFIGLKHHHAGYEQFGSGSGSGSGSGSTGGSRTGSGSGSGSGSGSPG

SEQ ID NO: 56 - protein, 975 aa, Artificial sequence
  Artificial sequence comprising at least one exosomal polypeptide and at least one Fc binding polypeptide
MDQARSAFSNLFGGEPLSYTRFSLARQVDGDNSHVEMKLAVDEEENADNNTKANVTKPKRCSGSICYGTIAVIVFFLIGFMIGYLGYCKGVEPKTECERLAGTESPVREEPGEDFPAARRLYWDDLKRKLSEKLDSTDFTGTIKLLNENSYVPREAGSQKDENLALYVENQFREFKLSKVWRDQHFVKIQVKDSAQNSVIIVDKNGRLVYLVENPGGYVAYSKAATVTGKLVHANFGTKKDFEDLYTPVNGSIVIVRAGKITFAEKVANAESLNAIGVLIYMDQTKFPIVNAELSFFGHAHLGTGDPYTPGFPSFNHTQFPPSRSSGLPNIPVQTISRAAAEKLFGNMEGDCPSDWKTDSTCRMVTSESKNVKLTVSNVLKEIKILNIFGVIKGFVEPDHYVVVGAQRDAWGPGAAKSGVGTALLLKLAQMFSDMVLKDGFQPSRSIIFASWSAGDFGSVGATEWLEGYLSSLHLKAFTYINLDKAVLGTSNFKVSASPLLYTLIEKTMQNVKHPVTGQFLYQDSNWASKVEKLTLDNAAFPFLAYSGIPAVSFCFCEDTDYPYLGTTMDTYKELIERIPELNKVARAAAEVAGQFVIKLTHDVELNLDYERYNSQLLSFVRDLNQYRADIKEMGLSLQWLYSARGDFFRATSRLTTDFGNAEKTDRFVMKKLNDRVMRVEYHFLSPYVSPKESPFRHVFWGSGSHTLPALLENLKLRKQNNGAFNETLFRNQLALATWTIQGAANALSGDVWDIDNEFGGGGSGGGGSQEGDFPMPFISAKSSPVIPLDGSVKIQCQAIREAYLTQLMIIKNSTYREIGRRLKFWNETDPEFVIDHMDANKAGRYQCQYRIGHYRFRYSDTLELVVTGLYGKPFLSADRGLVLMPGENISLTCSSAHIPFDRFSLAKEGELSLPQHQSGEHPANFSLGPVDLNVSGIYRCYGWYNRSPYLWSFPSNALELVVTDSIHQDYTTQN

SEQ ID NO: 57 - protein, 376 aa, Streptococcus pyogenes
MTRQQTKKNYSLRKLKTGTASVAVALTVLGAGFANQTTVKAEGAKIDWQEEYKKLDEDNAKLVEVVETTSLENEKLKSENEENKKNLDKLSKENQGKLEKLELDYLKKLDHEHKEHQKEQQEQEERQKNQEQLERKYQREVEKRYQEQLQKQQQLETEKQISEASRKSLSRDLEASRAAKKDLEAEHQKLEAEHQKLKEDKQISDASRQGLSRDLEASRAAKKELEANHQKLEAEHQKLKEDKQISDASRQGLSRDLEASRAAKKELEANHQKLEAEAKALKEQLAKQAEELAKLRAGKASDSQTPDTKPGNKAVPGKGQAPQAGTKPNQNKAPMKETKRQLPSTGETANPFFTAAALTVMATAGVAAVVKRKEEN

SEQ ID NO: 58 - protein, 450 aa, Staphylococcus aureus
MKKKNIYSIRKLGVGIASVTLGTLLISGGVTPAANAAQHDEAQQNAFYQVLNMPNLNADQRNGFIQSLKDDPSQSANVLGEAQKLNDSQAPKADAQQNNFNKDQQSAFYEILNMPNLNEAQRNGFIQSLKDDPSQSTNVLGEAKKLNESQAPKADNNFNKEQQNAFYEILNMPNLNEEQRNGFIQSLKDDPSQSANLLSEAKKLNESQAPKADNKFNKEQQNAFYEILHLPNLNEEQRNGFIQSLKDDPSVSKEILAEAKKLNDAQAPKEEDNKKPGKEDGNKPGKEDGNKPGKEDNKKPGKEDGNKPGKEDNNKPGKEDGNKPGKEDNNKPGKEDGNKPGKEDGNKPGKEDGNGVHVVKPGDTVNDIAKANGTTADKIAADNKLADKNMIKPGQELVVDKKQPANHADANKAQALPETGEENPFIGTTVFGGLSLALGAALLAGRRREL

SEQ ID NO: 59 - protein, 593 aa, Streptococcus sp
MEKEKKVKYFLRKSAFGLASVSAAFLVGSTVFAVDSPIEDTPIIRNGGELTNLLGNSETTLALRNEESATADLTAAAVADTVAAAAAENAGAAAWEAAAAADALAKAKADALKEFNKYGVSDYYKNLINNAKTVEGVKDLQAQVVESAKKARISEATDGLSDFLKSQTPAEDTVKSIELAEAKVLANRELDKYGVSDYHKNLINNAKTVEGVKDLQAQVVESAKKARISEATDGLSDFLKSQTPAEDTVKSIELAEAKVLANRELDKYGVSDYYKNLINNAKTVEGVKALIDEILAALPKTDTYKLILNGKTLKGETTTEAVDAATAEKVFKQYANDNGVDGEWTYDDATKTFTVTEKPEVIDASELTPAVTTYKLVINGKTLKGETTTEAVDAATAEKVFKQYANDNGVDGEWTYDDATKTFTVTEKPEVIDASELTPAVTTYKLVINGKTLKGETTTKAVDAETAEKAFKQYANDNGVDGVWTYDDATKTFTVTEMVTEVPGDAPTEPEKPEASIPLVPLTPATPIAKDDAKKDDTKKEDAKKPEAKKEDAKKAETLPTTGEGSNPFFTAAALAVMAGAGALAVASKRKED

SEQ ID NO: 60 - protein, 10 aa, Artifcial sequence
TWKTSRISIF

SEQ ID NO: 61 - protein, 13 aa, Artifcial sequence
DCAWHLGELVWCT

SEQ ID NO: 62 - protein, 10 aa, Artifcial sequence
FGRLVSSIRY

SEQ ID NO: 63 - protein, 12 aa, Artifcial sequence
EPIHRSTLTALL

SEQ ID NO: 64 - protein, 6 aa, Artifcial sequence
HWRGWV

SEQ ID NO: 65 - protein, 6 aa, Artifcial sequence
HYFKFD

SEQ ID NO: 66 - protein, 6 aa, Artifcial sequence
HFRRHL

SEQ ID NO: 67 - protein, 8 aa, Artifcial sequence
NKFRGKYK

SEQ ID NO: 68 - protein, 8 aa, Artifcial sequence
NARKFYKG

SEQ ID NO: 69 - protein, 8 aa, Artifcial sequence
FYWHCLDE

SEQ ID NO: 70 - protein, 8 aa, Artifcial sequence
FYCHWALE

SEQ ID NO: 71 - protein, 8 aa, Artifcial sequence
FYCHTIDE

SEQ ID NO: 72 - protein, 429 aa, Artifcial sequence
NAAQHDEAQQNAFYQVLNMPNLNADQRNGFIQSLKDDPSQSANVLGEAQKLNDSQAPKADAQQNNFNKDQQSAFYEILNMPNLNEAQRNGFIQSLKDDPSQSTNVLGEAKKLNESQAPKADNNFNKEQQNAFYEILNMPNLNEEQRNGFIQSLKDDPSQSANLLSEAKKLNESQAPKADNKFNKEQQNAFYEILHLPNLNEEQRNGFIQSLKDDPSQSANLLAEAKKLNDAQAPKADNKFNKEQQNAFYEILHLPNLTEEQRNGFIQSLKDDPSVSKEILAEAKKLNDAQAPKEEDSLEGSGSGTYKLILNGKTLKGETTTEAVDAATAEKVFKQYANDNGVDGEWTYDDATKTFTVTEKPEVIDASELTPAVTTYKLVINGKTLKGETTTKAVDAETAEKAFKQYANDNGVDGVWTYDDATKTFTVTE

SEQ ID NO: 73 - protein, 57 aa, Artifcial sequence
DNKFNKEQQNAFYEILHLPNLNEEQRNAFIQSLKDDPSQSANLLAEAKKLNDAQAPK

SEQ ID NO: 74 - protein, 114 aa, Artifcial sequence
DNKFNKEQQNAFYEILHLPNLNEEQRNAFIQSLKDDPSQSANLLAEAKKLNDAQAPKDNKFNKEQQNAFYEILHLPNLNEEQRNAFIQSLKDDPSQSANLLAEAKKLNDAQAPK

SEQ ID NO: 75 - protein, 665 aa, Artificial sequence
  Artificial sequence comprising at least one exosomal polypeptide and at least one Fc binding polypeptide
MGVEGCTKCIKYLLFVFNFVFWLAGGVILGVALWLRHDPQTTNLLYLELGDKPAPNTFYVGIYILIAVGAVMMFVGFLGCYGAIQESQCLLGTFFTCLVILFACEVAAGIWGFVNKDQIAKDVKQFYDQALQQAVVDDDANNAKAVVKTFHETLDCCGSSTLTALTTSNAAQHDEAQQNAFYQVLNMPNLNADQRNGFIQSLKDDPSQSANVLGEAQKLNDSQAPKADAQQNNFNKDQQSAFYEILNMPNLNEAQRNGFIQSLKDDPSQSTNVLGEAKKLNESQAPKADNNFNKEQQNAFYEILNMPNLNEEQRNGFIQSLKDDPSQSANLLSEAKKLNESQAPKADNKFNKEQQNAFYEILHLPNLNEEQRNGFIQSLKDDPSQSANLLAEAKKLNDAQAPKADNKFNKEQQNAFYEILHLPNLTEEQRNGFIQSLKDDPSVSKEILAEAKKLNDAQAPKEEDSLEGSGSGTYKLILNGKTLKGETTTEAVDAATAEKVFKQYANDNGVDGEWTYDDATKTFTVTEKPEVIDASELTPAVTTYKLVINGKTLKGETTTKAVDAETAEKAFKQYANDNGVDGVWTYDDATKTFTVTEVLKNNLCPSGSNIISNLFKEDCHQKIDDLFSGKLYLIGIAAIVVAVIMIFEMILSMVLCCGIRNSSVY

SEQ ID NO: 76 - protein, 342 aa, Artifical sequence
MPVKGGTKCIKYLLFGFNFIFWLAGIAVLAIGLWLRFDSQTKSIFEQETNNNNSSFYTGVYILIGAGALMMLVGFLGCCGAVQESQCMLGLFFGFLLVIFAIEIAAAIWGYSHKDEVIKEVQEFYKDTYNKLKTKDEPQRETLKAIHYALNCCGLAGGVEQFISDDNKFNKEQQNAFYEILHLPNLNEEQRNAFIQSLKDDPSQSANLLAEAKKLNDAQAPKDNKFNKEQQNAFYEILHLPNLNEEQRNAFIQSLKDDPSQSANLLAEAKKLNDAQAPKICPKKDVLETFTVKSCPDAIKEVFDNKFHIIGAVGIGIAVVMIFGMIFSMILCCAIRRNREMV

SEQ ID NO: 77 - protein, 296 aa, Staphylococcus aureus
NAAQHDEAQQNAFYQVLNMPNLNADQRNGFIQSLKDDPSQSANVLGEAQKLNDSQAPKADAQQNNFNKDQQSAFYEILNMPNLNEAQRNGFIQSLKDDPSQSTNVLGEAKKLNESQAPKADNNFNKEQQNAFYEILNMPNLNEEQRNGFIQSLKDDPSQSANLLSEAKKLNESQAPKADNKFNKEQQNAFYEILHLPNLNEEQRNGFIQSLKDDPSQSANLLAEAKKLNDAQAPKADNKFNKEQQNAFYEILHLPNLTEEQRNGFIQSLKDDPSVSKEILAEAKKLNDAQAPKEED

SEQ ID NO: 78 - protein, 125 aa, Streptococcus dysgalactiae
TYKLILNGKTLKGETTTEAVDAATAEKVFKQYANDNGVDGEWTYDDATKTFTVTEKPEVIDASELTPAVTTYKLVINGKTLKGETTTKAVDAETAEKAFKQYANDNGVDGVWTYDDATKTFTVTE

SEQ ID NO: 79 - protein, 404 aa, Mus musculus
MILTSFGDDMWLLTTLLLWVPVGGEVVNATKAVITLQPPWVSIFQKENVTLWCEGPHLPGDSSTQWFINGTAVQISTPSYSIPEASFQDSGEYRCQIGSSMPSDPVQLQIHNDWLLLQASRRVLTEGEPLALRCHGWKNKLVYNVVFYRNGKSFQFSSDSEVAILKTNLSHSGIYHCSGTGRHRYTSAGVSITVKELFTTPVLRASVSSPFPEGSLVTLNCETNLLLQRPGLQLHFSFYVGSKILEYRNTSSEYHIARAEREDAGFYWCEVATEDSSVLKRSPELELQVLGPQSSAPVWFHILFYLSVGIMFSLNTVLYVKIHRLQREKKYNLEVPLVSEQGKKANSFQQVRSDGVYEEVTATASQTTPKEAPDGPRSSVGDCGPEQPEPLPPSDSTGAQTSQS

SEQ ID NO: 80 - protein, 330 aa, Mus musculus
MESNWTVHVFSRTLCHMLLWTAVLNLAAGTHDLPKAVVKLEPPWIQVLKEDTVTLTCEGTHNPGNSSTQWFHNGRSIRSQVQASYTFKATVNDSGEYRCQMEQTRLSDPVDLGVISDWLLLQTPQLVFLEGETITLRCHSWRNKLLNRISFFHNEKSVRYHHYSSNFSIPKANHSHSGDYYCKGSLGRTLHQSKPVTITVQGPKSSRSLPVLTIVAAVTGIAVAAIVIILVSLVYLKKKQVPALPGNPDHREMGETLPEEVGEYRQPSGGSVPVSPGPPSGLEPTSSSPYNPPDLEEAAKTEAENTITYSLLKHPEALDEETEHDYQNHI

SEQ ID NO: 81 - protein, 261 aa, Mus musculus
MFQNAHSGSQWLLPPLTILLLFAFADRQSAALPKAVVKLDPPWIQVLKEDMVTLMCEGTHNPGNSSTQWFHNGRSIRSQVQASYTFKATVNDSGEYRCQMEQTRLSDPVDLGVISDWLLLQTPQRVFLEGETITLRCHSWRNKLLNRISFFHNEKSVRYHHYKSNFSIPKANHSHSGDYYCKGSLGSTQHQSKPVTITVQDPATTSSISLVWYHTAFSLVMCLLFAVDTGLYFYVRRNLQTPREYWRKSLSIRKHQAPQDK

SEQ ID NO: 82 - protein, 249 aa, Mus musculus
MWQLLLPTALVLTAFSGIQAGLQKAVVNLDPKWVRVLEEDSVTLRCQGTFSPEDNSIKWFHNESLIPHQDANYVIQSARVKDSGMYRCQTALSTISDPVQLEVHMGWLLLQTTKWLFQEGDPIHLRCHSWQNRPVRKVTYLQNGKGKKYFHENSELLIPKATHNDSGSYFCRGLIGHNNKSSASFRISLGDPGSPSMFPPWHQITFCLLIGLLFAIDTVLYFSVRRGLQSPVADYEEPKIQWSKEPQDK

SEQ ID NO: 83 - protein, 365 aa, Mus musculus
MGMPLPWALSLLLVLLPQTWGSETRPPLMYHLTAVSNPSTGLPSFWATGWLGPQQYLTYNSLRQEADPCGAWMWENQVSWYWEKETTDLKSKEQLFLEALKTLEKILNGTYTLQGLLGCELASDNSSVPTAVFALNGEEFMKFNPRIGNWTGEWPETEIVANLWMKQPDAARKESEFLLNSCPERLLGHLERGRRNLEWKEPPSMRLKARPGNSGSSVLTCAAFSFYPPELKFRFLRNGLASGSGNCSTGPNGDGSFHAWSLLEVKRGDEHHYQCQVEHEGLAQPLTVDLDSSARSSVPVVGIVLGLLLVVVAIAGGVLLWGRMRSGLPAPWLSLSGDDSGDLLPGGNLPPEAEPQGANAFPATS